European Patent Specification EP 3 131 588 B1, published November 5, 2025. Title: IMIDE-BASED MODULATORS OF PROTEOLYSIS AND ASSOCIATED METHODS OF USE. Applicant: Arvinas, Inc. Crew, Andrew Crews, Craig Wang, Jing Dong, Hanqing Jin, Meizhong Qian, Yimin Chen, Xin Ferraro, Caterina Siu, Kam. The sequence listing filed with the application follows.

SEQUENCE LISTING (5 sequences)

SEQ ID NO: 1 - DNA, 41 bp, Artificial Sequence
  Primer Sequence
gtgccgcgtggctccatggccggcgaaggagatcagcagga

SEQ ID NO: 2 - DNA, 41 bp, Artificial Sequence
  Primer Sequence
gcttcctttcgggcttattacaagcaaagtattactttgtc

SEQ ID NO: 3 - DNA, 50 bp, Artificial Sequence
  Primer Sequence
tcgggcgcggctctcggtccgaaaaggatgtcgtacaactacgtggtaac

SEQ ID NO: 4 - DNA, 61 bp, Artificial Sequence
  Primer Sequence
gcttcctttcgggcttatttttcgaactgcgggtggctccaatggatccgagttagctcct

SEQ ID NO: 5 - DNA, 61 bp, Artificial Sequence
  Primer Sequence
gcttcctttcgggcttacttatcgtcatcgtccttgtagtccaagcaaagtattactttgt